European Patent Application EP 4 549 587 A1, published May 7, 2025. Title: METHOD FOR THE DIAGNOSIS OF A CANCER WITH CHROMATIN-BOIUND MDM2. Applicant: INSTITUT REGIONAL DU CANCER DE MONTPELLIER. The sequence listing filed with the application follows.

SEQUENCE LISTING (3 sequences)

SEQ ID NO: 1 - DNA, 20 bp, synthetic construct
  source 1..20: mol_type = other DNA
aattgagatagggtcctgcc

SEQ ID NO: 2 - DNA, 20 bp, synthetic construct
  source 1..20: mol_type = other DNA
tggcatgcacctgttattcc

SEQ ID NO: 3 - DNA, 23 bp, synthetic construct
  source 1..23: mol_type = other DNA
ttccaggctggagtgcagtgatg